European Patent Specification EP 4 032 973 B1, published July 19, 2023. Title: Modified T cells for adoptive immunotherapy. Applicant: Guizhou Sinorda Biotechnology CO., Ltd. The sequence listing filed with the application follows.

SEQUENCE LISTING (6 sequences)

SEQ ID NO: 1 - RNA, 21 nt, Artificial Sequence
  siRNA
ucucccgacaggcucauuutt

SEQ ID NO: 2 - RNA, 21 nt, Artificial Sequence
  siRNA
aaaugagccugucgggagatt

SEQ ID NO: 3 - RNA, 21 nt, Artificial Sequence
  siRNA
ggagaacuugcucaacacatt

SEQ ID NO: 4 - RNA, 21 nt, Artificial Sequence
  siRNA
uguguugagcaaguucucctt

SEQ ID NO: 5 - RNA, 21 nt, Artificial Sequence
  siRNA
aggcccaggaguccaauuatt

SEQ ID NO: 6 - RNA, 21 nt, Artificial Sequence
  siRNA
uaauuggacuccugggccutt